European Patent Specification EP 3 594 240 B1, published December 6, 2023. Title: ANTI-TRANSFERRIN RECEPTOR ANTIBODIES AND METHODS OF USE. Applicant: F. Hoffmann-La Roche AG. The sequence listing filed with the application follows.

SEQUENCE LISTING (175 sequences)

SEQ ID NO: 1 - protein, 760 aa, Homo sapiens
MMDQARSAFSNLFGGEPLSYTRFSLARQVDGDNSHVEMKLAVDEEENADNNTKANVTKPKRCSGSICYGTIAVIVFFLIGFMIGYLGYCKGVEPKTECERLAGTESPVREEPGEDFPAARRLYWDDLKRKLSEKLDSTDFTSTIKLLNENSYVPREAGSQKDENLALYVENQFREFKLSKVWRDQHFVKIQVKDSAQNSVIIVDKNGRLVYLVENPGGYVAYSKAATVTGKLVHANFGTKKDFEDLYTPVNGSIVIVRAGKITFAEKVANAESLNAIGVLIYMDQTKFPIVNAELSFFGHAHLGTGDPYTPGFPSFNHTQFPPSRSSGLPNIPVQTISRAAAEKLFGNMEGDCPSDWKTDSTCRMVTSESKNVKLTVSNVLKEIKILNIFGVIKGFVEPDHYVVVGAQRDAWGPGAAKSGVGTALLLKLAQMFSDMVLKDGFQPSRSIIFASWSAGDFGSVGATEWLEGYLSSLHLKAFTYINLDKAVLGTSNFKVSASPLLYTLIEKTMQNVKHPVTGQFLYQDSNWASKVEKLTLDNAAFPFLAYSGIPAVSFCFCEDTDYPYLGTTMDTYKELIERIPELNKVARAAAEVAGQFVIKLTHDVELNLDYERYNSQLLSFVRDLNQYRADIKEMGLSLQWLYSARGDFFRATSRLTTDFGNAEKTDRFVMKKLNDRVMRVEYHFLSPYVSPKESPFRHVFWGSGSHTLPALLENLKLRKQNNGAFNETLFRNQLALATWTIQGAANALSGDVWDIDNEF

SEQ ID NO: 2 - protein, 760 aa, Macaca mulatta
MMDQARSAFSNLFGGEPLSYTRFSLARQVDGDNSHVEMKLGVDEEENTDNNTKPNGTKPKRCGGNICYGTIAVIIFFLIGFMIGYLGYCKGVEPKTECERLAGTESPAREEPEEDFPAAPRLYWDDLKRKLSEKLDTTDFTSTIKLLNENLYVPREAGSQKDENLALYIENQFREFKLSKVWRDQHFVKIQVKDSAQNSVIIVDKNGGLVYLVENPGGYVAYSKAATVTGKLVHANFGTKKDFEDLDSPVNGSIVIVRAGKITFAEKVANAESLNAIGVLIYMDQTKFPIVKADLSFFGHAHLGTGDPYTPGFPSFNHTQFPPSQSSGLPNIPVQTISRAAAEKLFGNMEGDCPSDWKTDSTCKMVTSENKSVKLTVSNVLKETKILNIFGVIKGFVEPDHYVVVGAQRDAWGPGAAKSSVGTALLLKLAQMFSDMVLKDGFQPSRSIIFASWSAGDFGSVGATEWLEGYLSSLHLKAFTYINLDKAVLGTSNFKVSASPLLYTLIEKTMQDVKHPVTGRSLYQDSNWASKVEKLTLDNAAFPFLAYSGIPAVSFCFCEDTDYPYLGTTMDTYKELVERIPELNKVARAAAEVAGQFVIKLTHDTELNLDYERYNSQLLLFLRDLNQYRADVKEMGLSLQWLYSARGDFFRATSRLTTDFRNAEKRDKFVMKKLNDRVMRVEYYFLSPYVSPKESPFRHVFWGSGSHTLSALLESLKLRRQNNSAFNETLFRNQLALATWTIQGAANALSGDVWDIDNEF

SEQ ID NO: 3 - protein, 763 aa, Mus musculus
MMDQARSAFSNLFGGEPLSYTRFSLARQVDGDNSHVEMKLAADEEENADNNMKASVRKPKRFNGRLCFAAIALVIFFLIGFMSGYLGYCKRVEQKEECVKLAETEETDKSETMETEDVPTSSRLYWADLKTLLSEKLNSIEFADTIKQLSQNTYTPREAGSQKDESLAYYIENQFHEFKFSKVWRDEHYVKIQVKSSIGQNMVTIVQSNGNLDPVESPEGYVAFSKPTEVSGKLVHANFGTKKDFEELSYSVNGSLVIVRAGEITFAEKVANAQSFNAIGVLIYMDKNKFPVVEADLALFGHAHLGTGDPYTPGFPSFNHTQFPPSQSSGLPNIPVQTISRAAAEKLFGKMEGSCPARWNIDSSCKLELSQNQNVKLIVKNVLKERRILNIFGVIKGYEEPDRYVVVGAQRDALGAGVAAKSSVGTGLLLKLAQVFSDMISKDGFRPSRSIIFASWTAGDFGAVGATEWLEGYLSSLHLKAFTYINLDKVVLGTSNFKVSASPLLYTLMGKIMQDVKHPVDGKSLYRDSNWISKVEKLSFDNAAYPFLAYSGIPAVSFCFCEDADYPYLGTRLDTYEALTQKVPQLNQMVRTAAEVAGQLIIKLTHDVELNLDYEMYNSKLLSFMKDLNQFKTDIRDMGLSLQWLYSARGDYFRATSRLTTDFHNAEKTNRFVMREINDRIMKVEYHFLSPYVSPRESPFRHIFWGSGSHTLSALVENLKLRQKNITAFNETLFRNQLALATWTIQGVANALSGDIWNIDNEF

SEQ ID NO: 4 - protein, 111 aa, Artificial Sequence
  source: /note="Description of Artificial Sequence: Synthetic polypeptide"
DIVLTQSPASLAVSLGQRATISCRASESVDDYGNSFMHWYQQKPGQPPKLLIYRASNLESGIPARFSGSGSRTDFTLTINPVEADDVATYYCQQSNEAPPTFGGGTKLEIR

SEQ ID NO: 5 - protein, 111 aa, Artificial Sequence
  source: /note="Description of Artificial Sequence: Synthetic polypeptide"
DIVLTQSPASLAVSLGQRATISCRASESVDSYGNSFMHWYQQKPGQPPKLLIYRASNLESGIPARFSGSGSRTDFTLTINPVEADDVATYYCQQSNEGPPTFGGGTKLEIK

SEQ ID NO: 6 - protein, 111 aa, Artificial Sequence
  source: /note="Description of Artificial Sequence: Synthetic polypeptide"
DIVLTQSPASLAVSLGQRATISCRASESVDSYGPSFMHWYQQKPGQPPKLLIYRASNLESGIPARFSGSGSRTDFTLTINPVEADDVATYYCQHSNEDPPTFGGGTRLEIK

SEQ ID NO: 7 - protein, 119 aa, Artificial Sequence
  source: /note="Description of Artificial Sequence: Synthetic polypeptide"
QVQLQQSGPELVRPGVSVKISCKGSGYTFTDYAMHWVKQSHAKSLEWIGGISTYFGRTNYNQKFKGRATMTVDKSSSTAYMELARLTSEDSALYYCARGLSGNYVMDYWGQGTSVTVSS

SEQ ID NO: 8 - protein, 119 aa, Artificial Sequence
  source: /note="Description of Artificial Sequence: Synthetic polypeptide"
QVQLQQSGPELVRPGVSVKISCKGSGYTFTDYGMHWVKQSHAKSLEWIGVISPYSGRTNYNQNFKGKATMTVDKSSSTAYLELARLTSEDSAIYYCARGLSGNYVVDYWGQGTSVTVSS

SEQ ID NO: 9 - protein, 119 aa, Artificial Sequence
  source: /note="Description of Artificial Sequence: Synthetic polypeptide"
QVQLQQSGPELVRPGVSVKISCKGSGYTVTDYAMHWVKQSHAKSLEWIGVISFYSGKTNYNQKFMGKATMTVDKSSSTAYMELARLTSEDSAIYYCARGLSGNYVMDYWGQGTSVTVSS

SEQ ID NO: 10 - protein, 119 aa, Artificial Sequence
  source: /note="Description of Artificial Sequence: Synthetic polypeptide"
QVQLQQSGPELVRPGVAVKISCKGSGYKFIDYGMHWVKQSHTKSLQWIGVISPYSGKTNYSQKFKGKATMTVDKSSSTAYMELARLTSEDSAIYYCARGLSGNFVMDFWGQGTSVTVSS

SEQ ID NO: 11 - protein, 107 aa, Artificial Sequence
  source: /note="Description of Artificial Sequence: Synthetic polypeptide"
DIQMTQSPASLSVSVGETVTITCRASDNLYSNLAWYQQKQGKSPQLLVYDATNLADGVPSRFSGSGSGTQYSLKINSLQSEDFGTYYCQHFWGTPLTFGAGTKLELK

SEQ ID NO: 12 - protein, 107 aa, Artificial Sequence
  source: /note="Description of Artificial Sequence: Synthetic polypeptide"
DIQLTQTPASLSVSVGETVTITCRASENIYSNLAWYQQKQGKSPQLLVYAATDLADGVPSRFRGSGSGTQYSLKINSLQSEDFGSYYCQHFWGTPLTFGAGTKLELI

SEQ ID NO: 13 - protein, 107 aa, Artificial Sequence
  source: /note="Description of Artificial Sequence: Synthetic polypeptide"
DIQMTQSPASLSVSVGETVTITCRASDNIYSNLAWYQQKQGKSPQLLVYAATNLADGVPSRFSGSGSGTQYSLKINSLQSEDFGSYYCQHFWGTPLMFGSGTKLELK

SEQ ID NO: 14 - protein, 107 aa, Artificial Sequence
  source: /note="Description of Artificial Sequence: Synthetic polypeptide"
DIQMTQSPASLSVSVGETVTITCRASDNIYSNLAWYQQKQGKSPQLLVYAVTNLADGVPSRFSGSGSGTQYSLKINSLQSEDFGSYYCQHFWGTPLTFGAGTKLELK

SEQ ID NO: 15 - protein, 116 aa, Artificial Sequence
  source: /note="Description of Artificial Sequence: Synthetic polypeptide"
QVQLQQPGAELVKPGASVKLSCKASGYTFTSYWMHWVKQRPGQGLEWIGEINPTNGRTNYIEKFKSKATLTVDKSSSTAYMQLSSLTSEDSAVYYCARGTRAYHYWGQGTSVTVSS

SEQ ID NO: 16 - protein, 116 aa, Artificial Sequence
  source: /note="Description of Artificial Sequence: Synthetic polypeptide"
QVQLQQPGAELVRPGAAVKLSCKASGYTFTSYWMHWVKQRPGQGLEWIGEINPTNGRTNYNENFKSKATLTVDKSSSTAYMQLSSLTSEDSAVYYCARGTRAYHFWGQGTSVTVSS

SEQ ID NO: 17 - protein, 116 aa, Artificial Sequence
  source: /note="Description of Artificial Sequence: Synthetic polypeptide"
QVQLQQPGAELVKPGASVKLSCKASGYTFASYWMHWVKQRPGQGLEWIGEINPINGRTNYSEKFKKKATLTVDKSSSTAYMQLSSLTSEDSAVYYCARGTRAYHYWGQGTSVTVSS

SEQ ID NO: 18 - protein, 116 aa, Artificial Sequence
  source: /note="Description of Artificial Sequence: Synthetic polypeptide"
QVQLQQPGAELVKPGASVKLSCKASGYTFTSYWMHWVKQRPGQGLEWIGEINPSNGRTNYNETFKSKATLTVDKSSSTAYMQLSSLTSEDSAVYYCARGTRAYHYWGQGTSVTVSS

SEQ ID NO: 19 - protein, 107 aa, Artificial Sequence
  source: /note="Description of Artificial Sequence: Synthetic polypeptide"
DVQITQSPSYLTASPGETITINCRASKSISKYLAWYQEKPGKTNKLLIYSGSTLQSGIPSRFSGSGSGTDFTLTISNLEPEDFAMYYCQQHNEYPWTFGGGTKLEIK

SEQ ID NO: 20 - protein, 122 aa, Artificial Sequence
  source: /note="Description of Artificial Sequence: Synthetic polypeptide"
DVQLQESGPGLVKPSQSLSLTCTVTGNSITSEYAWNWIRQFPGNKLEWMGYISYSGTTSYNPSLKSRISITRDTSKNQLFLQLNSVTTEDTATYFCARYGYGNPATRYFDVWGAGTTVTVSS

SEQ ID NO: 21 - protein, 111 aa, Artificial Sequence
  source: /note="Description of Artificial Sequence: Synthetic polypeptide"
DIVLTQSPASLAVSLGQRATISCRARQSVSTSSYSFMHWYRQKAGQPPKLLIKYASIQESGVPARFSGSGSGTDFTLNILPVEEEDTATYYCQHTWEIPFTFGSGTKLEIK

SEQ ID NO: 22 - protein, 111 aa, Artificial Sequence
  source: /note="Description of Artificial Sequence: Synthetic polypeptide"
DIVLTQSPASLAVSLGQRATISCRARQSVSTSSYSFMHWYQQKPGQPPKLLIKYASIQESGVPARFSGSGSGTDFTLNILPVEEEDTATYYCQHTWEIPFTFGSGTNLEIK

SEQ ID NO: 23 - protein, 108 aa, Artificial Sequence
  source: /note="Description of Artificial Sequence: Synthetic polypeptide"
QIVLTQSPAIMSASLGGRVTMTCTTSSSVPSSYFHWYQQKPGSSPKLWIYSTSNLASGVPARFSGSGSGTSYSLTISSMEAEDAATYYCHQYHRSPFTFGSGTKLEIK

SEQ ID NO: 24 - protein, 107 aa, Artificial Sequence
  source: /note="Description of Artificial Sequence: Synthetic polypeptide"
DIQMTQTTSSLSASLGDRVTINCRAGQDITNYLNWFQQKPDGTVKLLIYYTSRLHSGVPSRFSGSGSGTDYSLTITNLEQEDIATYFCQQANTLPYTFGGGTKLEIK

SEQ ID NO: 25 - protein, 120 aa, Artificial Sequence
  source: /note="Description of Artificial Sequence: Synthetic polypeptide"
QVQLQQPGSELVRPGASVKLSCKASGYTFTSYWMHWVKQRHGQGLEWIGNIYPGSGSTKYDERFKSKGTLTVDTSSSTAYMHLSSLTSEDSAVYYCTRGGYDSRAWFAYWGQGTLVTVSA

SEQ ID NO: 26 - protein, 120 aa, Artificial Sequence
  source: /note="Description of Artificial Sequence: Synthetic polypeptide"
QVQLQQPGSELVRPGASVKLSCKASGYTFTSYWMHWVKQRHGQGLEWIGNIYPGSGSTKYDEKFKSKGTLTVDTSSSTAYMHLSSLTSEDSAVYYCTRGGYDSRAWFAHWGQGTLVTVSA

SEQ ID NO: 27 - protein, 124 aa, Artificial Sequence
  source: /note="Description of Artificial Sequence: Synthetic polypeptide"
EVKLVESGGGLVQPGGFLKLSCATSGFTFSDYYMYWVRQTPEKRLEWVASISNGGDNTYYPDTVKGRFTISRDNAKNTLYLQMSRLKSEDTAMYYCARQGALYDGYYRGAMDYWGQGTSVTVSS

SEQ ID NO: 28 - protein, 121 aa, Artificial Sequence
  source: /note="Description of Artificial Sequence: Synthetic polypeptide"
QVQLQQSGAELMKPGASVKISCKAAGYTFSNYWIEWVKQRPGHGLEWIGEILPGSGSTKYNEKFKGKATFTADTSSNTAYMQLSSLTSEDSAVYYCARRGGYGYDGEFAYWGQGTLVTVSA

SEQ ID NO: 29 - protein, 15 aa, Artificial Sequence
  source: /note="Description of Artificial Sequence: Synthetic peptide"
RASESVDSYGNSFMH

SEQ ID NO: 30 - protein, 7 aa, Artificial Sequence
  source: /note="Description of Artificial Sequence: Synthetic peptide"
RASNLES

SEQ ID NO: 31 - protein, 9 aa, Artificial Sequence
  source: /note="Description of Artificial Sequence: Synthetic peptide"
QQSNEAPPT

SEQ ID NO: 32 - protein, 5 aa, Artificial Sequence
  source: /note="Description of Artificial Sequence: Synthetic peptide"
DYAMH

SEQ ID NO: 33 - protein, 17 aa, Artificial Sequence
  source: /note="Description of Artificial Sequence: Synthetic peptide"
GISTYFGRTNYNQKFKG

SEQ ID NO: 34 - protein, 10 aa, Artificial Sequence
  source: /note="Description of Artificial Sequence: Synthetic peptide"
GLSGNYVMDY

SEQ ID NO: 35 - protein, 15 aa, Artificial Sequence
  source: /note="Description of Artificial Sequence: Synthetic peptide"
RASESVDSYGNSFMH

SEQ ID NO: 36 - protein, 9 aa, Artificial Sequence
  source: /note="Description of Artificial Sequence: Synthetic peptide"
QQSNEGPPT

SEQ ID NO: 37 - protein, 5 aa, Artificial Sequence
  source: /note="Description of Artificial Sequence: Synthetic peptide"
DYGMH

SEQ ID NO: 38 - protein, 17 aa, Artificial Sequence
  source: /note="Description of Artificial Sequence: Synthetic peptide"
VISPYSGRTNYNQNFKG

SEQ ID NO: 39 - protein, 10 aa, Artificial Sequence
  source: /note="Description of Artificial Sequence: Synthetic peptide"
GLSGNYVVDY

SEQ ID NO: 40 - protein, 17 aa, Artificial Sequence
  source: /note="Description of Artificial Sequence: Synthetic peptide"
VISFYSGKTNYNQKFMG

SEQ ID NO: 41 - protein, 15 aa, Artificial Sequence
  source: /note="Description of Artificial Sequence: Synthetic peptide"
RASESVDSYGNSFMH

SEQ ID NO: 42 - protein, 9 aa, Artificial Sequence
  source: /note="Description of Artificial Sequence: Synthetic peptide"
QHSNEDPPT

SEQ ID NO: 43 - protein, 17 aa, Artificial Sequence
  source: /note="Description of Artificial Sequence: Synthetic peptide"
VISPYSGKTNYSQKFKG

SEQ ID NO: 44 - protein, 10 aa, Artificial Sequence
  source: /note="Description of Artificial Sequence: Synthetic peptide"
GLSGNFVMDF

SEQ ID NO: 45 - protein, 15 aa, Artificial Sequence
  source: /note="Description of Artificial Sequence: Synthetic peptide"
  VARIANT (8)..(8): /replace="Asp"
  VARIANT (11)..(11): /replace="Pro"
  misc_feature (1)..(15): /note="Variant residues given in the sequence have no preference with respect to those in the annotations for variant positions"
RASESVDSYGNSFMH

SEQ ID NO: 46 - protein, 9 aa, Artificial Sequence
  source: /note="Description of Artificial Sequence: Synthetic peptide"
  VARIANT (2)..(2): /replace="His"
  VARIANT (6)..(6): /replace="Gly" or "Asp"
  misc_feature (1)..(9): /note="Variant residues given in the sequence have no preference with respect to those in the annotations for variant positions"
QQSNEAPPT

SEQ ID NO: 47 - protein, 5 aa, Artificial Sequence
  source: /note="Description of Artificial Sequence: Synthetic peptide"
  VARIANT (3)..(3): /replace="Gly"
  misc_feature (1)..(5): /note="Variant residues given in the sequence have no preference with respect to those in the annotations for variant positions"
DYAMH

SEQ ID NO: 48 - protein, 17 aa, Artificial Sequence
  source: /note="Description of Artificial Sequence: Synthetic peptide"
  VARIANT (1)..(1): /replace="Val"
  VARIANT (4)..(4): /replace="Phe" or "Pro"
  VARIANT (6)..(6): /replace="Ser"
  VARIANT (8)..(8): /replace="Lys"
  VARIANT (12)..(12): /replace="Ser"
  VARIANT (14)..(14): /replace="Asn"
  VARIANT (16)..(16): /replace="Met"
  misc_feature (1)..(17): /note="Variant residues given in the sequence have no preference with respect to those in the annotations for variant positions"
GISTYFGRTNYNQKFKG

SEQ ID NO: 49 - protein, 10 aa, Artificial Sequence
  source: /note="Description of Artificial Sequence: Synthetic peptide"
  VARIANT (6)..(6): /replace="Phe"
  VARIANT (8)..(8): /replace="Val"
  VARIANT (10)..(10): /replace="Phe"
  misc_feature (1)..(10): /note="Variant residues given in the sequence have no preference with respect to those in the annotations for variant positions"
GLSGNYVMDY

SEQ ID NO: 50 - protein, 11 aa, Artificial Sequence
  source: /note="Description of Artificial Sequence: Synthetic peptide"
RASDNLYSNLA

SEQ ID NO: 51 - protein, 7 aa, Artificial Sequence
  source: /note="Description of Artificial Sequence: Synthetic peptide"
DATNLAD

SEQ ID NO: 52 - protein, 9 aa, Artificial Sequence
  source: /note="Description of Artificial Sequence: Synthetic peptide"
QHFWGTPLT

SEQ ID NO: 53 - protein, 5 aa, Artificial Sequence
  source: /note="Description of Artificial Sequence: Synthetic peptide"
SYWMH

SEQ ID NO: 54 - protein, 17 aa, Artificial Sequence
  source: /note="Description of Artificial Sequence: Synthetic peptide"
EINPTNGRTNYIEKFKS

SEQ ID NO: 55 - protein, 7 aa, Artificial Sequence
  source: /note="Description of Artificial Sequence: Synthetic peptide"
GTRAYHY

SEQ ID NO: 56 - protein, 11 aa, Artificial Sequence
  source: /note="Description of Artificial Sequence: Synthetic peptide"
RASENIYSNLA

SEQ ID NO: 57 - protein, 7 aa, Artificial Sequence
  source: /note="Description of Artificial Sequence: Synthetic peptide"
AATDLAD

SEQ ID NO: 58 - protein, 17 aa, Artificial Sequence
  source: /note="Description of Artificial Sequence: Synthetic peptide"
EINPTNGRTNYNENFKS

SEQ ID NO: 59 - protein, 7 aa, Artificial Sequence
  source: /note="Description of Artificial Sequence: Synthetic peptide"
GTRAYHF

SEQ ID NO: 60 - protein, 11 aa, Artificial Sequence
  source: /note="Description of Artificial Sequence: Synthetic peptide"
RASDNIYSNLA

SEQ ID NO: 61 - protein, 7 aa, Artificial Sequence
  source: /note="Description of Artificial Sequence: Synthetic peptide"
AATNLAD

SEQ ID NO: 62 - protein, 9 aa, Artificial Sequence
  source: /note="Description of Artificial Sequence: Synthetic peptide"
QHFWGTPLM

SEQ ID NO: 63 - protein, 17 aa, Artificial Sequence
  source: /note="Description of Artificial Sequence: Synthetic peptide"
EINPINGRTNYSEKFKK

SEQ ID NO: 64 - protein, 7 aa, Artificial Sequence
  source: /note="Description of Artificial Sequence: Synthetic peptide"
AVTNLAD

SEQ ID NO: 65 - protein, 17 aa, Artificial Sequence
  source: /note="Description of Artificial Sequence: Synthetic peptide"
EINPSNGRTNYNETFKS

SEQ ID NO: 66 - protein, 11 aa, Artificial Sequence
  source: /note="Description of Artificial Sequence: Synthetic peptide"
  VARIANT (4)..(4): /replace="Asp"
  VARIANT (6)..(6): /replace="Ile"
  misc_feature (1)..(11): /note="Variant residues given in the sequence have no preference with respect to those in the annotations for variant positions"
RASENLYSNLA

SEQ ID NO: 67 - protein, 7 aa, Artificial Sequence
  source: /note="Description of Artificial Sequence: Synthetic peptide"
  VARIANT (1)..(1): /replace="Ala"
  VARIANT (2)..(2): /replace="Val"
  VARIANT (4)..(4): /replace="Asp"
  misc_feature (1)..(7): /note="Variant residues given in the sequence have no preference with respect to those in the annotations for variant positions"
DATNLAD

SEQ ID NO: 68 - protein, 9 aa, Artificial Sequence
  source: /note="Description of Artificial Sequence: Synthetic peptide"
  VARIANT (9)..(9): /replace="Met"
  misc_feature (1)..(9): /note="Variant residues given in the sequence have no preference with respect to those in the annotations for variant positions"
QHFWGTPLT

SEQ ID NO: 69 - protein, 17 aa, Artificial Sequence
  source: /note="Description of Artificial Sequence: Synthetic peptide"
  VARIANT (5)..(5): /replace="Ile" or "Ser"
  VARIANT (12)..(12): /replace="Asn" or "Ser"
  VARIANT (14)..(14): /replace="Asn" or "Thr"
  VARIANT (17)..(17): /replace="Lys"
  misc_feature (1)..(17): /note="Variant residues given in the sequence have no preference with respect to those in the annotations for variant positions"
EINPTNGRTNYIEKFKS

SEQ ID NO: 70 - protein, 7 aa, Artificial Sequence
  source: /note="Description of Artificial Sequence: Synthetic peptide"
  VARIANT (7)..(7): /replace="Phe"
  misc_feature (1)..(7): /note="Variant residues given in the sequence have no preference with respect to those in the annotations for variant positions"
GTRAYHY

SEQ ID NO: 71 - protein, 11 aa, Artificial Sequence
  source: /note="Description of Artificial Sequence: Synthetic peptide"
RASKSISKYLA

SEQ ID NO: 72 - protein, 7 aa, Artificial Sequence
  source: /note="Description of Artificial Sequence: Synthetic peptide"
SGSTLQS

SEQ ID NO: 73 - protein, 9 aa, Artificial Sequence
  source: /note="Description of Artificial Sequence: Synthetic peptide"
QQHNEYPWT

SEQ ID NO: 74 - protein, 6 aa, Artificial Sequence
  source: /note="Description of Artificial Sequence: Synthetic peptide"
SEYAWN

SEQ ID NO: 75 - protein, 16 aa, Artificial Sequence
  source: /note="Description of Artificial Sequence: Synthetic peptide"
YISYSGTTSYNPSLKS

SEQ ID NO: 76 - protein, 13 aa, Artificial Sequence
  source: /note="Description of Artificial Sequence: Synthetic peptide"
YGYGNPATRYFDV

SEQ ID NO: 77 - protein, 15 aa, Artificial Sequence
  source: /note="Description of Artificial Sequence: Synthetic peptide"
RARQSVSTSSYSFMH

SEQ ID NO: 78 - protein, 7 aa, Artificial Sequence
  source: /note="Description of Artificial Sequence: Synthetic peptide"
YASIQES

SEQ ID NO: 79 - protein, 9 aa, Artificial Sequence
  source: /note="Description of Artificial Sequence: Synthetic peptide"
QHTWEIPFT

SEQ ID NO: 80 - protein, 5 aa, Artificial Sequence
  source: /note="Description of Artificial Sequence: Synthetic peptide"
SYWMH

SEQ ID NO: 81 - protein, 17 aa, Artificial Sequence
  source: /note="Description of Artificial Sequence: Synthetic peptide"
NIYPGSGSTKYDERFKS

SEQ ID NO: 82 - protein, 11 aa, Artificial Sequence
  source: /note="Description of Artificial Sequence: Synthetic peptide"
GGYDSRAWFAY

SEQ ID NO: 83 - protein, 17 aa, Artificial Sequence
  source: /note="Description of Artificial Sequence: Synthetic peptide"
NIYPGSGSTKYDEKFKS

SEQ ID NO: 84 - protein, 11 aa, Artificial Sequence
  source: /note="Description of Artificial Sequence: Synthetic peptide"
GGYDSRAWFAH

SEQ ID NO: 85 - protein, 12 aa, Artificial Sequence
  source: /note="Description of Artificial Sequence: Synthetic peptide"
TTSSSVPSSYFH

SEQ ID NO: 86 - protein, 7 aa, Artificial Sequence
  source: /note="Description of Artificial Sequence: Synthetic peptide"
STSNLAS

SEQ ID NO: 87 - protein, 9 aa, Artificial Sequence
  source: /note="Description of Artificial Sequence: Synthetic peptide"
HQYHRSPFT

SEQ ID NO: 88 - protein, 5 aa, Artificial Sequence
  source: /note="Description of Artificial Sequence: Synthetic peptide"
DYYMY

SEQ ID NO: 89 - protein, 17 aa, Artificial Sequence
  source: /note="Description of Artificial Sequence: Synthetic peptide"
SISNGGDNTYYPDTVKG

SEQ ID NO: 90 - protein, 15 aa, Artificial Sequence
  source: /note="Description of Artificial Sequence: Synthetic peptide"
QGALYDGYYRGAMDY

SEQ ID NO: 91 - protein, 11 aa, Artificial Sequence
  source: /note="Description of Artificial Sequence: Synthetic peptide"
RAGQDITNYLN

SEQ ID NO: 92 - protein, 7 aa, Artificial Sequence
  source: /note="Description of Artificial Sequence: Synthetic peptide"
YTSRLHS

SEQ ID NO: 93 - protein, 9 aa, Artificial Sequence
  source: /note="Description of Artificial Sequence: Synthetic peptide"
QQANTLPYT

SEQ ID NO: 94 - protein, 5 aa, Artificial Sequence
  source: /note="Description of Artificial Sequence: Synthetic peptide"
NYWIE

SEQ ID NO: 95 - protein, 17 aa, Artificial Sequence
  source: /note="Description of Artificial Sequence: Synthetic peptide"
EILPGSGSTKYNEKFKG

SEQ ID NO: 96 - protein, 12 aa, Artificial Sequence
  source: /note="Description of Artificial Sequence: Synthetic peptide"
RGGYGYDGEFAY

SEQ ID NO: 97 - protein, 15 aa, Artificial Sequence
  source: /note="Description of Artificial Sequence: Synthetic peptide"
  VARIANT (1)..(1): /replace="Thr"
  VARIANT (2)..(2): /replace="Thr"
  VARIANT (3)..(3): /replace="Ser" or "Gly"
  VARIANT (4)..(4): /replace="Ser"
  VARIANT (5)..(8): /replace=" "
  VARIANT (9)..(9): /replace="Val" or "Asp"
  VARIANT (10)..(10): /replace="Pro" or "Ile"
  VARIANT (11)..(11): /replace="Ser" or "Thr"
  VARIANT (12)..(12): /replace="Asn"
  VARIANT (13)..(13): /replace="Tyr"
  VARIANT (14)..(14): /replace="Phe" or "Leu"
  VARIANT (15)..(15): /replace="Asn"
  misc_feature (1)..(15): /note="Variant residues given in the sequence have no preference with respect to those in the annotations for variant positions"
RARQSVSTSSYSFMH

SEQ ID NO: 98 - protein, 7 aa, Artificial Sequence
  source: /note="Description of Artificial Sequence: Synthetic peptide"
  VARIANT (1)..(1): /replace="Ser"
  VARIANT (2)..(2): /replace="Thr"
  VARIANT (4)..(4): /replace="Asn" or "Arg"
  VARIANT (5)..(5): /replace="Leu"
  VARIANT (6)..(6): /replace="Ala" or "His"
  misc_feature (1)..(7): /note="Variant residues given in the sequence have no preference with respect to those in the annotations for variant positions"
YASIQES

SEQ ID NO: 99 - protein, 9 aa, Artificial Sequence
  source: /note="Description of Artificial Sequence: Synthetic peptide"
  VARIANT (1)..(1): /replace="His"
  VARIANT (2)..(2): /replace="Gln"
  VARIANT (3)..(3): /replace="Tyr" or "Ala"
  VARIANT (4)..(4): /replace="His" or "Asn"
  VARIANT (5)..(5): /replace="Arg" or "Thr"
  VARIANT (6)..(6): /replace="Ser" or "Leu"
  VARIANT (8)..(8): /replace="Tyr"
  misc_feature (1)..(9): /note="Variant residues given in the sequence have no preference with respect to those in the annotations for variant positions"
QHTWEIPFT

SEQ ID NO: 100 - protein, 5 aa, Artificial Sequence
  source: /note="Description of Artificial Sequence: Synthetic peptide"
  VARIANT (1)..(1): /replace="Asp" or "Asn"
  VARIANT (3)..(3): /replace="Tyr"
  VARIANT (4)..(4): /replace="Ile"
  VARIANT (5)..(5): /replace="Tyr" or "Glu"
  misc_feature (1)..(5): /note="Variant residues given in the sequence have no preference with respect to those in the annotations for variant positions"
SYWMH

SEQ ID NO: 101 - protein, 17 aa, Artificial Sequence
  source: /note="Description of Artificial Sequence: Synthetic peptide"
  VARIANT (1)..(1): /replace="Ser" or "Glu"
  VARIANT (3)..(3): /replace="Ser" or "Leu"
  VARIANT (4)..(4): /replace="Asn"
  VARIANT (6)..(6): /replace="Gly"
  VARIANT (7)..(7): /replace="Asp"
  VARIANT (8)..(8): /replace="Asn"
  VARIANT (10)..(10): /replace="Tyr"
  VARIANT (12)..(12): /replace="Pro" or "Asn"
  VARIANT (13)..(13): /replace="Asp"
  VARIANT (14)..(14): /replace="Lys" or "Thr"
  VARIANT (15)..(15): /replace="Val"
  VARIANT (17)..(17): /replace="Gly"
  misc_feature (1)..(17): /note="Variant residues given in the sequence have no preference with respect to those in the annotations for variant positions"
NIYPGSGSTKYDERFKS

SEQ ID NO: 102 - protein, 15 aa, Artificial Sequence
  source: /note="Description of Artificial Sequence: Synthetic peptide"
  VARIANT (1)..(1): /replace="Gln" or "Arg"
  VARIANT (3)..(3): /replace="Ala" or "Gly"
  VARIANT (4)..(4): /replace="Leu" or "Tyr"
  VARIANT (5)..(5): /replace="Tyr" or "Gly"
  VARIANT (6)..(6): /replace="Asp" or "Tyr"
  VARIANT (7)..(7): /replace="Gly" or "Asp"
  VARIANT (8)..(8): /replace="Tyr" or "Gly"
  VARIANT (9)..(9): /replace="Tyr" or "Glu"
  VARIANT (10)..(10): /replace="Phe" or " "
  VARIANT (11)..(13): /replace=" "
  VARIANT (14)..(14): /replace="Asp"
  VARIANT (15)..(15): /replace="His"
  misc_feature (1)..(15): /note="Variant residues given in the sequence have no preference with respect to those in the annotations for variant positions"
GGYDSRAWFRGAMAY

SEQ ID NO: 103 - protein, 107 aa, Homo sapiens
DIQMTQSPSSLSASVGDRVTITCRASQGISNSLAWYQQKPGKAPKLLLYAASRLESGVPSRFSGSGSGTDYTLTISSLQPEDFATYYCQQYYSTPYTFGQGTKLEIK

SEQ ID NO: 104 - protein, 107 aa, Mus musculus; identical to SEQ ID NO: 11

SEQ ID NO: 105 - protein, 107 aa, Artificial Sequence
  source: /note="Description of Artificial Sequence: Synthetic polypeptide"
DIQMTQSPSSLSASVGDRVTITCRASDNLYSNLAWYQQKPGKSPKLLVYDATNLADGVPSRFSGSGSGTDYTLTISSLQPEDFATYYCQHFWGTPLTFGQGTKVEIK

SEQ ID NO: 106 - protein, 112 aa, Homo sapiens
QVQLVQSGAEVKKPGASVKVSCKASGYTFTSYAMHWVRQAPGQRLEWMGWINAGNGNTKYSQKFQGRVTITRDTSASTAYMELSSLRSEDTAVYYCARFDVWGQGTMVTVSS

SEQ ID NO: 107 - protein, 116 aa, Mus musculus; identical to SEQ ID NO: 15

SEQ ID NO: 108 - protein, 116 aa, Artificial Sequence
  source: /note="Description of Artificial Sequence: Synthetic polypeptide"
EVQLVQSGAEVKKPGASVKVSCKASGYTFTSYWMHWVRQAPGQRLEWIGEINPTNGRTNYIEKFKSRATLTVDKSASTAYMELSSLRSEDTAVYYCARGTRAYHYWGQGTMVTVSS

SEQ ID NO: 109 - protein, 113 aa, Homo sapiens
DIVMTQSPDSLAVSLGERATINCKSSQSVLYSSNNKNYLAWYQQKPGQPPKLLIYWASTRESGVPDRFSGSGSGTDFTLTISSLQAEDVAVYYCQQYYSTPYTFGQGTKLEIK

SEQ ID NO: 110 - protein, 111 aa, Mus musculus; identical to SEQ ID NO: 5

SEQ ID NO: 111 - protein, 111 aa, Artificial Sequence
  source: /note="Description of Artificial Sequence: Synthetic polypeptide"
DIVMTQSPDSLAVSLGERATINCRASESVDSYGNSFMHWYQQKPGQPPKLLIYRASNLESGVPDRFSGSGSRTDFTLTISSLQAEDVAVYYCQQSNEAPPTFGQGTKLEIK

SEQ ID NO: 112 - protein, 112 aa, Homo sapiens
QVQLVQSGAEVKKPGASVKVSCKASGYTFTGYYMHWVRQAPGQGLEWMGWINPNSGGTNYAQKFQGRVTMTRDTSISTAYMELSRLRSDDTAVYYCARMDYWGQGTTVTVSS

SEQ ID NO: 113 - protein, 119 aa, Mus musculus; identical to SEQ ID NO: 7

SEQ ID NO: 114 - protein, 119 aa, Artificial Sequence
  source: /note="Description of Artificial Sequence: Synthetic polypeptide"
EVQLVQSGAEVKKPGASVKVSCKGSGYTFTDYAMHWVRQAPGQGLEWMGGISTYFGRTNYNQKFKGRVTMTVDTSISTAYMELSRLRSDDTAVYYCARGLSGNYVMDYWGQGTTVTVSS

SEQ ID NO: 115 - protein, 113 aa, Homo sapiens
DIVMTQSPDSLAVSLGERATINCKSSQSVLYSSNNKNYLAWYQQKPGQPPKLLIYWASTRESGVPDRFSGSGSGTDFTLTISSLQAEDVAVYYCQQYYSTPFTFGQGTKVEIK

SEQ ID NO: 116 - protein, 111 aa, Mus musculus; identical to SEQ ID NO: 21

SEQ ID NO: 117 - protein, 111 aa, Artificial Sequence
  source: /note="Description of Artificial Sequence: Synthetic polypeptide"
DIVMTQSPDSLAVSLGERATINCRARQSVSTSSYSFMHWYQQPAGQPPKLLIKYASIQESGVPDRFSGSGSGTDFTLTISSLQAEDVAVYYCQHTWEIPFTFGQGTKVEIK

SEQ ID NO: 118 - protein, 112 aa, Homo sapiens
EVQLVQSGAEVKKPGASVKVSCKASGYTFTSYYIHWVRQAPGQGLEWIGWINPGSGNTNYAQKFQGRVTITRDTSTSTAYLELSSLRSEDTAVYYCARFDYWGQGTLVTVSS

SEQ ID NO: 119 - protein, 120 aa, Mus musculus; identical to SEQ ID NO: 25

SEQ ID NO: 120 - protein, 120 aa, Artificial Sequence
  source: /note="Description of Artificial Sequence: Synthetic polypeptide"
EVQLVQSGAEVKKPGASVKVSCKASGYTFTSYWMHWVRQAPGQGLEWIGNIYPGSGSTKYDERFKSRVTITVDTSTSTAYLELSSLRSEDTAVYYCTRGGYDSRAWFAYWGQGTLVTVSS

SEQ ID NO: 121 - protein, 107 aa, Homo sapiens
DIQLTQSPSFLSASVGDRVTITCRASQGISSYLAWYQQKPGKAPKLLIYAASTLQSGVPSRFSGSGSGTEFTLTISSLQPEDFATYYCQQLNSYPWTFGQGTKVEIK

SEQ ID NO: 122 - protein, 107 aa, Mus musculus; identical to SEQ ID NO: 19

SEQ ID NO: 123 - protein, 107 aa, Artificial Sequence
  source: /note="Description of Artificial Sequence: Synthetic polypeptide"
DIQMTQSPSSLSASVGDRVTITCRASKSISKYLAWYQQKPGKTNKLLLYSGSTLQSGVPSRFSGSGSGTDYTLTISSLQPEDFATYYCQQHNEYPWTFGQGTKVEIK

SEQ ID NO: 124 - protein, 111 aa, Homo sapiens
QVQLQESGPGLVKPSETLSLTCTVSGGSISSYYWSWIRQPPGKGLEWIGYIYYSGSTNYNPSLKSRVTISVDTSKNQFSLKLSSVTAADTAVYYCARMDVWGKGTTVTVSS

SEQ ID NO: 125 - protein, 122 aa, Mus musculus; identical to SEQ ID NO: 20

SEQ ID NO: 126 - protein, 122 aa, Artificial Sequence
  source: /note="Description of Artificial Sequence: Synthetic polypeptide"
EVQLVESGPGLVKPSETLSLTCTVSGNSITSEYAWNWIRQPPGKGLEWIGYISYSGTTSYNPSLKSRVTISRDTSKNQLSLKLSSVTAADTAVYYCARYGYGNPATRYFDVWGQGTLVTVSS

SEQ ID NO: 127 - protein, 9 aa, Artificial Sequence
  source: /note="Description of Artificial Sequence: Synthetic peptide"
QQSNEAPPT

SEQ ID NO: 128 - protein, 9 aa, Artificial Sequence
  source: /note="Description of Artificial Sequence: Synthetic peptide"
QHFWGTPLT

SEQ ID NO: 129 - protein, 7 aa, Artificial Sequence
  source: /note="Description of Artificial Sequence: Synthetic peptide"
GTRAYHY

SEQ ID NO: 130 - protein, 9 aa, Artificial Sequence
  source: /note="Description of Artificial Sequence: Synthetic peptide"
QQSNEAPPT

SEQ ID NO: 131 - protein, 10 aa, Artificial Sequence
  source: /note="Description of Artificial Sequence: Synthetic peptide"
GLSGNYVMDY

SEQ ID NO: 132 - protein, 108 aa, Artificial Sequence
  source: /note="Description of Artificial Sequence: Synthetic polypeptide"
DIQMTQSPSSLSASVGDRVTITCRASQDVSTAVAWYQQKPGKAPKLLIYSASFLYSGVPSRFSGSGSGTDFTLTISSLQPEDFATYYCQQSYTTPPTFGQGTKVEIKR

SEQ ID NO: 133 - protein, 108 aa, Artificial Sequence
  source: /note="Description of Artificial Sequence: Synthetic polypeptide"
DIQMTQSPSSLSASVGDRVTITCRASQDVSTAVAWYQQKPGKAPKLLIYSASFLYSGVPSRFSGSGSGTDFTLTISSLQPEDFATYYCQQFPTYLPTFGQGTKVEIKR

SEQ ID NO: 134 - protein, 108 aa, Artificial Sequence
  source: /note="Description of Artificial Sequence: Synthetic polypeptide"
DIQMTQSPSSLSASVGDRVTITCRASQDVSTAVAWYQQKPGKAPKLLIYSASFLYSGVPSRFSGSGSGTDFTLTISSLQPEDFATYYCQQGYNDPPTFGQGTKVEIKR

SEQ ID NO: 135 - protein, 108 aa, Artificial Sequence
  source: /note="Description of Artificial Sequence: Synthetic polypeptide"
DIQMTQSPSSLSASVGDRVTITCRASQDVSTAVAWYQQKPGKAPKLLIYSASFLYSGVPSRFSGSGSGTDFTLTISSLQPEDFATYYCQQSSTDPTTFGQGTKVEIKR

SEQ ID NO: 136 - protein, 108 aa, Artificial Sequence
  source: /note="Description of Artificial Sequence: Synthetic polypeptide"
DIQMTQSPSSLSASVGDRVTITCRASQVVANSLAWYQQKPGKAPKLLIYLASFLYSGVPSRFSGSGSGTDFTLTISSLQPEDFATYYCQQDATSPPTFGQGTKVEIKR

SEQ ID NO: 137 - protein, 108 aa, Artificial Sequence
  source: /note="Description of Artificial Sequence: Synthetic polypeptide"
DIQMTQSPSSLSASVGDRVTITCRASQDVSTAVAWYQQKPGKAPKLLIYSASFLYSGVPSRFSGSGSGTDFTLTISSLQPEDFATYYCQQYATDPPTFGQGTKVEIKR

SEQ ID NO: 138 - protein, 119 aa, Artificial Sequence
  source: /note="Description of Artificial Sequence: Synthetic polypeptide"
EVQLVESGGGLVQPGGSLRLSCAASGFTFSGYAIHWVRQAPGKGLEWVGWISPAGGSTDYADSVKGRFTISADTSKNTAYLQMNSLRAEDTAVYYCARGPFSPWVMDYWGQGTLVTVSS

SEQ ID NO: 139 - protein, 119 aa, Artificial Sequence
  source: /note="Description of Artificial Sequence: Synthetic polypeptide"
EVQLVESGGGLVQPGGSLRLSCAASGFTFLGYGIHWVRQAPGKGLEWVGWISPAGGSTDYADSVKGRFTISADTSKNTAYLQMNSLRAEDTAVYYCARGPFSPWVMDYWGQGTLVTVSS

SEQ ID NO: 140 - protein, 108 aa, Artificial Sequence
  source: /note="Description of Artificial Sequence: Synthetic polypeptide"
DIQMTQSPSSLSASVGDRVTITCRASQSVSSAVAWYQQKPGKAPKLLIYSASSLYSGVPSRFSGSGSGTDFTLTISSLQPEDFATYYCQQYSYSPFTFGQGTKVEIKR

SEQ ID NO: 141 - protein, 108 aa, Artificial Sequence
  source: /note="Description of Artificial Sequence: Synthetic polypeptide"
DIQMTQSPSSLSASVGDRVTITCRASQSVSSAVAWYQQKPGKAPKLLISWASWLYSGVPSRFSGSGSGTDFTLTISSLQPEDFATYYCQQYSYSPFTFGQGTKVEIKR

SEQ ID NO: 142 - protein, 108 aa, Artificial Sequence
  source: /note="Description of Artificial Sequence: Synthetic polypeptide"
DIQMTQSPSSLSASVGDRVTITCRASQSVSSAVAWYQQKPGKAPKLLIWYASWLYSGVPSRFSGSGSGTDFTLTISSLQPEDFATYYCQQYSYSPFTFGQGTKVEIKR

SEQ ID NO: 143 - protein, 108 aa, Artificial Sequence
  source: /note="Description of Artificial Sequence: Synthetic polypeptide"
DIQMTQSPSSLSASVGDRVTITCRASQSVSSAVAWYQQKPGKAPKLLIWWASSLYSGVPSRFSGSGSGTDFTLTISSLQPEDFATYYCQQYSYSPFTFGQGTKVEIKR

SEQ ID NO: 144 - protein, 126 aa, Artificial Sequence
  source: /note="Description of Artificial Sequence: Synthetic polypeptide"
EVQLVESGGGLVQPGGSLRLSCAASGFNFYYSSIHWVRQAPGKGLEWVASISPYSGYTSYADSVKGRFTISADTSKNTAYLQMNSLRAEDTAVYYCARQPTHYYYYAKGYKAMDYWGQGTLVTVSS

SEQ ID NO: 145 - protein, 438 aa, Artificial Sequence
  source: /note="Description of Artificial Sequence: Synthetic polypeptide"
EVQLVESGGGLVQPGGSLRLSCAASGFTFSSYGMSWVRQAPGKGLELVASINSNGGSTYYPDSVKGRFTISRDNAKNSLYLQMNSLRAEDTAVYYCASGDYWGQGTTVTVSSASTKGPSVFPLAPCSRSTSESTAALGCLVKDYFPEPVTVSWNSGALTSGVHTFPAVLQSSGLYSLSSVVTVPSSSLGTKTYTCNVDHKPSNTKVDKRVESKYGPPCPPCPAPEFLGGPSVFLFPPKPKDTLMISRTPEVTCVVVDVSQEDPEVQFNWYVDGVEVHNAKTKPREEQFNSTYRVVSVLTVLHQDWLNGKEYKCKVSNKGLPSSIEKTISKAKGQPREPQVYTLPPSQEEMTKNQVSLTCLVKGFYPSDIAVEWESNGQPENNYKTTPPVLDSDGSFFLYSRLTVDKSRWQEGNVFSCSVMHEALHNHYTQKSLSLSLG

SEQ ID NO: 146 - protein, 219 aa, Artificial Sequence
  source: /note="Description of Artificial Sequence: Synthetic polypeptide"
DIVMTQSPLSLPVTPGEPASISCRSSQSLVYSNGDTYLHWYLQKPGQSPQLLIYKVSNRFSGVPDRFSGSGSGTDFTLKISRVEAEDVGVYYCSQSTHVPWTFGQGTKVEIKRTVAAPSVFIFPPSDEQLKSGTASVVCLLNNFYPREAKVQWKVDNALQSGNSQESVTEQDSKDSTYSLSSTLTLSKADYEKHKVYACEVTHQGLSSPVTKSFNRGEC

SEQ ID NO: 147 - protein, 10 aa, Artificial Sequence
  source: /note="Description of Artificial Sequence: Synthetic peptide"
GYTFTSYWMH

SEQ ID NO: 148 - protein, 10 aa, Artificial Sequence
  source: /note="Description of Artificial Sequence: Synthetic peptide"
GYTFTDYAMH

SEQ ID NO: 149 - protein, 9 aa, Artificial Sequence
  source: /note="Description of Artificial Sequence: Synthetic peptide"
GYTFSYWMH

SEQ ID NO: 150 - protein, 107 aa, Artificial Sequence; identical to SEQ ID NO: 105
  source: /note="Description of Artificial Sequence: Synthetic polypeptide"

SEQ ID NO: 151 - protein, 107 aa, Artificial Sequence
  source: /note="Description of Artificial Sequence: Synthetic polypeptide"
DIQMTQSPSSLSASVGDRVTITCRASDNLYSNLAWYQQKPGKSPKLLVYDATNLADGVPSRFSGSGSGTDYTLTISSLQPEDFATYYCQHFAGTPLTFGQGTKVEIK

SEQ ID NO: 152 - protein, 116 aa, Artificial Sequence; identical to SEQ ID NO: 108
  source: /note="Description of Artificial Sequence: Synthetic polypeptide"

SEQ ID NO: 153 - protein, 116 aa, Artificial Sequence
  source: /note="Description of Artificial Sequence: Synthetic polypeptide"
EVQLVQSGAEVKKPGASVKVSCKASGYTFTSYWMHWVRQAPGQRLEWIGEIAPTNGRTNYIEKFKSRATLTVDKSASTAYMELSSLRSEDTAVYYCARGTRAYHYWGQGTMVTVSS

SEQ ID NO: 154 - protein, 116 aa, Artificial Sequence
  source: /note="Description of Artificial Sequence: Synthetic polypeptide"
EVQLVQSGAEVKKPGASVKVSCKASGYTFTSYWMHWVRQAPGQRLEWIGEINPANGRTNYIEKFKSRATLTVDKSASTAYMELSSLRSEDTAVYYCARGTRAYHYWGQGTMVTVSS

SEQ ID NO: 155 - protein, 9 aa, Artificial Sequence
  source: /note="Description of Artificial Sequence: Synthetic peptide"
QHFAGTPLT

SEQ ID NO: 156 - protein, 17 aa, Artificial Sequence
  source: /note="Description of Artificial Sequence: Synthetic peptide"
EIAPTNGRTNYIEKFKS

SEQ ID NO: 157 - protein, 17 aa, Artificial Sequence
  source: /note="Description of Artificial Sequence: Synthetic peptide"
EINPANGRTNYIEKFKS

SEQ ID NO: 158 - protein, 214 aa, Artificial Sequence
  source: /note="Description of Artificial Sequence: Synthetic polypeptide"
DIQMTQSPSSLSASVGDRVTITCRASDNLYSNLAWYQQKPGKSPKLLVYDATNLADGVPSRFSGSGSGTDYTLTISSLQPEDFATYYCQHFWGTPLTFGQGTKVEIKRTVAAPSVFIFPPSDEQLKSGTASVVCLLNNFYPREAKVQWKVDNALQSGNSQESVTEQDSKDSTYSLSSTLTLSKADYEKHKVYACEVTHQGLSSPVTKSFNRGEC

SEQ ID NO: 159 - protein, 446 aa, Artificial Sequence
  source: /note="Description of Artificial Sequence: Synthetic polypeptide"
EVQLVQSGAEVKKPGASVKVSCKASGYTFTSYWMHWVRQAPGQRLEWIGEINPTNGRTNYIEKFKSRATLTVDKSASTAYMELSSLRSEDTAVYYCARGTRAYHYWGQGTMVTVSSASTKGPSVFPLAPSSKSTSGGTAALGCLVKDYFPEPVTVSWNSGALTSGVHTFPAVLQSSGLYSLSSVVTVPSSSLGTQTYICNVNHKPSNTKVDKKVEPKSCDKTHTCPPCPAPELLGGPSVFLFPPKPKDTLMISRTPEVTCVVVAVSHEDPEVKFNWYVDGVEVHNAKTKPREEQYGSTYRVVSVLTVLHQDWLNGKEYKCKVSNKALPAPIEKTISKAKGQPREPQVYTLPPSREEMTKNQVSLSCAVKGFYPSDIAVEWESNGQPENNYKTTPPVLDSDGSFFLVSKLTVDKSRWQQGNVFSCSVMHEALHNHYTQKSLSLSPGK

SEQ ID NO: 160 - protein, 108 aa, Artificial Sequence
  source: /note="Description of Artificial Sequence: Synthetic polypeptide"
DIQMTQSPSSLSASVGDRVTITCRASDNLYSNLAWYQQKPGKSPKLLVYDATNLADGVPSRFSGSGSGTDYTLTISSLQPEDFATYYCQHFAGTPLTFGQGTKVEIKR

SEQ ID NO: 161 - protein, 15 aa, Artificial Sequence
  source: /note="Description of Artificial Sequence: Synthetic peptide"
RASESVDDYGNSFMH

SEQ ID NO: 162 - protein, 15 aa, Artificial Sequence
  source: /note="Description of Artificial Sequence: Synthetic peptide"
RASESVDSYGPSFMH

SEQ ID NO: 163 - protein, 112 aa, Artificial Sequence
  source: /note="Description of Artificial Sequence: Synthetic polypeptide"
DIQMTQSPASLSVSVGETVTITCRASDNLYSNLAWYQQKQGKSPQLLVYDATNLADGVPSRFSGSGSGTQYSLKINSLQSEDFGTYYCQHFWGTPLTFGAGTKLELKRADAA

SEQ ID NO: 164 - protein, 125 aa, Artificial Sequence
  source: /note="Description of Artificial Sequence: Synthetic polypeptide"
QVQLQQPGAELVKPGASVKLSCKASGYTFTSYWMHWVKQRPGQGLEWIGEINPTNGRTNYIEKFKSKATLTVDKSSSTAYMQLSSLTSEDSAVYYCARGTRAYHYWGQGTSVTVSSAKTTAPSVY

SEQ ID NO: 165 - protein, 113 aa, Artificial Sequence
  source: /note="Description of Artificial Sequence: Synthetic polypeptide"
DIQLTQTPASLSVSVGETVTITCRASENIYSNLAWYQQKQGKSPQLLVYAATDLADGVPSRFRGSGSGTQYSLKINSLQSEDFGSYYCQHFWGTPLTFGAGTKLELIRADAAP

SEQ ID NO: 166 - protein, 125 aa, Artificial Sequence
  source: /note="Description of Artificial Sequence: Synthetic polypeptide"
QVQLQQPGAELVRPGAAVKLSCKASGYTFTSYWMHWVKQRPGQGLEWIGEINPTNGRTNYNENFKSKATLTVDKSSSTAYMQLSSLTSEDSAVYYCARGTRAYHFWGQGTSVTVSSAKTTAPSVY

SEQ ID NO: 167 - protein, 113 aa, Artificial Sequence
  source: /note="Description of Artificial Sequence: Synthetic polypeptide"
DIQMTQSPASLSVSVGETVTITCRASDNIYSNLAWYQQKQGKSPQLLVYAATNLADGVPSRFSGSGSGTQYSLKINSLQSEDFGSYYCQHFWGTPLMFGSGTKLELKRADAAP

SEQ ID NO: 168 - protein, 125 aa, Artificial Sequence
  source: /note="Description of Artificial Sequence: Synthetic polypeptide"
QVQLQQPGAELVKPGASVKLSCKASGYTFASYWMHWVKQRPGQGLEWIGEINPINGRTNYSEKFKKKATLTVDKSSSTAYMQLSSLTSEDSAVYYCARGTRAYHYWGQGTSVTVSSAKTTAPSVY

SEQ ID NO: 169 - protein, 119 aa, Artificial Sequence
  source: /note="Description of Artificial Sequence: Synthetic polypeptide"
QVQLQQPGAELVKPGASVKLSCKASGYTFTSYWMHWVKQRPGQGLEWIGEINPSNGRTNYNETFKSKATLTVDKSSSTAYMQLSSLTSEDSAVYYCARGTRAYHYWGQGTSVTVSSAKT

SEQ ID NO: 170 - protein, 113 aa, Artificial Sequence
  source: /note="Description of Artificial Sequence: Synthetic polypeptide"
DVQITQSPSYLTASPGETITINCRASKSISKYLAWYQEKPGKTNKLLIYSGSTLQSGIPSRFSGSGSGTDFTLTISNLEPEDFAMYYCQQHNEYPWTFGGGTKLEIKRADAAP

SEQ ID NO: 171 - protein, 131 aa, Artificial Sequence
  source: /note="Description of Artificial Sequence: Synthetic polypeptide"
DVQLQESGPGLVKPSQSLSLTCTVTGNSITSEYAWNWIRQFPGNKLEWMGYISYSGTTSYNPSLKSRISITRDTSKNQLFLQLNSVTTEDTATYFCARYGYGNPATRYFDVWGAGTTVTVSSAKTTPPSVY

SEQ ID NO: 172 - protein, 123 aa, Artificial Sequence
  source: /note="Description of Artificial Sequence: Synthetic polypeptide"
QVQLQQPGSELVRPGASVKLSCKASGYTFTSYWMHWVKQRHGQGLEWIGNIYPGSGSTKYDERFKSKGTLTVDTSSSTAYMHLSSLTSEDSAVYYCTRGGYDSRAWFAYWGQGTLVTVSAAKT

SEQ ID NO: 173 - protein, 123 aa, Artificial Sequence
  source: /note="Description of Artificial Sequence: Synthetic polypeptide"
QVQLQQPGSELVRPGASVKLSCKASGYTFTSYWMHWVKQRHGQGLEWIGNIYPGSGSTKYDEKFKSKGTLTVDTSSSTAYMHLSSLTSEDSAVYYCTRGGYDSRAWFAHWGQGTLVTVSAAKT

SEQ ID NO: 174 - protein, 127 aa, Artificial Sequence
  source: /note="Description of Artificial Sequence: Synthetic polypeptide"
EVKLVESGGGLVQPGGFLKLSCATSGFTFSDYYMYWVRQTPEKRLEWVASISNGGDNTYYPDTVKGRFTISRDNAKNTLYLQMSRLKSEDTAMYYCARQGALYDGYYRGAMDYWGQGTSVTVSSAKT

SEQ ID NO: 175 - protein, 124 aa, Artificial Sequence
  source: /note="Description of Artificial Sequence: Synthetic polypeptide"
QVQLQQSGAELMKPGASVKISCKAAGYTFSNYWIEWVKQRPGHGLEWIGEILPGSGSTKYNEKFKGKATFTADTSSNTAYMQLSSLTSEDSAVYYCARRGGYGYDGEFAYWGQGTLVTVSAAKT